European Patent Specification EP 3 280 271 B1, published February 26, 2025. Title: ANIMAL FEED COMPOSITIONS AND METHODS OF USE. Applicant: SYNGENTA PARTICIPATIONS AG Iragavarapu, Tammiraj Kumar Witherspoon, David. The sequence listing filed with the application follows.

SEQUENCE LISTING (5 sequences)

SEQ ID NO: 1 - protein, 436 aa, Artificial
  Synthetic
MAKYLELEEGGVIMQAFYWDVPSGGIWWDTIRQKIPEWYDAGISAIWIPPASKGMSGGYSMGYDPYDYFDLGEYYQKGTVETRFGSKQELINMINTAHAYGIKVIADIVINHRAGGDLEWNPFVGDYTWTDFSKVASGKYTANYLDFHPNELHAGDSGTFGGYPDICHDKSWDQYWLWASQESYAAYLRSIGIDAWRFDYVKGYGAWVVKDWLNWWGGWAVGEYWDTNVDALLNWAYSSGAKVFDFPLYYKMDAAFDNKNIPALVEALKNGGTVVSRDPFKAVTFVANHDTDIIWNKYPAYAFILTYEGQPTIFYRDYEEWLNKDKLKNLIWIHDNLAGGSTSIVYYDSDEMIFVRNGYGSKPGLITYINLGSSKVGRWVYVPKFAGACIHEYTGNLGGWVDKYVYSSGWVYLEAPAYDPANGQYGYSVWSYCGVG

SEQ ID NO: 2 - DNA, 1308 bp, Artificial
  Synthetic
atggccaagtacctggagctggaggagggcggcgtgatcatgcaggcgttctactgggacgtcccgagcggaggcatctggtgggacaccatccgccagaagatccccgagtggtacgacgccggcatctccgcgatctggataccgccagcttccaagggcatgtccgggggctactcgatgggctacgacccgtacgactacttcgacctcggcgagtactaccagaagggcacggtggagacgcgcttcgggtccaagcaggagctcatcaacatgatcaacacggcgcacgcctacggcatcaaggtcatcgcggacatcgtgatcaaccacagggccggcggcgacctggagtggaacccgttcgtcggcgactacacctggacggacttctccaaggtcgcctccggcaagtacaccgccaactacctcgacttccaccccaacgagctgcacgcgggcgactccggcacgttcggcggctacccggacatctgccacgacaagtcctgggaccagtactggctctgggcctcgcaggagtcctacgcggcctacctgcgctccatcggcatcgacgcgtggcgcttcgactacgtcaagggctacggggcctgggtggtcaaggactggctcaactggtggggcggctgggcggtgggcgagtactgggacaccaacgtcgacgcgctgctcaactgggcctactcctccggcgccaaggtgttcgacttccccctgtactacaagatggacgcggccttcgacaacaagaacatcccggcgctcgtcgaggccctgaagaacggcggcacggtggtctcccgcgacccgttcaaggccgtgaccttcgtcgccaaccacgacacggacatcatctggaacaagtacccggcgtacgccttcatcctcacctacgagggccagcccacgatcttctaccgcgactacgaggagtggctgaacaaggacaagctcaagaacctgatctggattcacgacaacctcgcgggcggctccactagtatcgtgtactacgactccgacgagatgatcttcgtccgcaacggctacggctccaagcccggcctgatcacgtacatcaacctgggctcctccaaggtgggccgctgggtgtacgtcccgaagttcgccggcgcgtgcatccacgagtacaccggcaacctcggcggctgggtggacaagtacgtgtactcctccggctgggtctacctggaggccccggcctacgaccccgccaacggccagtacggctactccgtgtggtcctactgcggcgtcggc

SEQ ID NO: 3 - DNA, 2223 bp, Artificial
  Synthetic
atggccaagtacctggagctggaggagggcggcgtgatcatgcaggcgttctactgggacgtcccgagcggaggcatctggtgggacaccatccgccagaagatccccgagtggtacgacgccggcatctccgcgatctggataccgccagcttccaagggcatgtccgggggctactcgatgggctacgacccgtacgactacttcgacctcggcgagtactaccagaagggcacggtggagacgcgcttcgggtccaagcaggagctcatcaacatgatcaacacggcgcacgcctacggcatcaaggtcatcgcggacatcgtgatcaaccacagggccggcggcgacctggagtggaacccgttcgtcggcgactacacctggacggacttctccaaggtcgcctccggcaagtacaccgccaactacctcgacttccaccccaacgagctgcacgcgggcgactccggcacgttcggcggctacccggacatctgccacgacaagtcctgggaccagtactggctctgggcctcgcaggagtcctacgcggcctacctgcgctccatcggcatcgacgcgtggcgcttcgactacgtcaagggctacggggcctgggtggtcaaggactggctcaactggtggggcggctgggcggtgggcgagtactgggacaccaacgtcgacgcgctgctcaactgggcctactcctccggcgccaaggtgttcgacttccccctgtactacaagatggacgcggccttcgacaacaagaacatcccggcgctcgtcgaggccctgaagaacggcggcacggtggtctcccgcgacccgttcaaggccgtgaccttcgtcgccaaccacgacacggacatcatctggaacaagtacccggcgtacgccttcatcctcacctacgagggccagcccacgatcttctaccgcgactacgaggagtggctgaacaaggacaagctcaagaacctgatctggattcacgacaacctcgcgggcggctccactagtatcgtgtactacgactccgacgagatgatcttcgtccgcaacggctacggctccaagcccggcctgatcacgtacatcaacctgggctcctccaaggtgggccgctgggtgtacgtcccgaagttcgccggcgcgtgcatccacgagtacaccggcaacctcggcggctgggtggacaagtacgtgtactcctccggctgggtctacctggaggccccggcctacgaccccgccaacggccagtacggctactccgtgtggtcctactgcggcgtcggcacatcgattgctggcatcctcgaggccgacagggtcctcaccgtcagcccctactacgccgaggagctcatctccggcatcgccaggggctgcgagctcgacaacatcatgcgcctcaccggcatcaccggcatcgtcaacggcatggacgtcagcgagtgggaccccagcagggacaagtacatcgccgtgaagtacgacgtgtcgacggccgtggaggccaaggcgctgaacaaggaggcgctgcaggcggaggtcgggctcccggtggaccggaacatcccgctggtggcgttcatcggcaggctggaagagcagaagggccccgacgtcatggcggccgccatcccgcagctcatggagatggtggaggacgtgcagatcgttctgctgggcacgggcaagaagaagttcgagcgcatgctcatgagcgccgaggagaagttcccaggcaaggtgcgcgccgtggtcaagttcaacgcggcgctggcgcaccacatcatggccggcgccgacgtgctcgccgtcaccagccgcttcgagccctgcggcctcatccagctgcaggggatgcgatacggaacgccctgcgcctgcgcgtccaccggtggactcgtcgacaccatcatcgaaggcaagaccgggttccacatgggccgcctcagcgtcgactgcaacgtcgtggagccggcggacgtcaagaaggtggccaccaccttgcagcgcgccatcaaggtggtcggcacgccggcgtacgaggagatggtgaggaactgcatgatccaggatctctcctggaagggccctgccaagaactgggagaacgtgctgctcagcctcggggtcgccggcggcgagccaggggttgaaggcgaggagatcgcgccgctcgccaaggagaacgtggccgcgccc

SEQ ID NO: 4 - DNA, 3285 bp, Aspergillus shirousami
gccaccccggccgactggcgctcccagtccatctacttcctcctcaccgaccgcttcgcccgcaccgacggctccaccaccgccacctgcaacaccgccgaccagaagtactgcggcggcacctggcagggcatcatcgacaagctcgactacatccagggcatgggcttcaccgccatctggatcaccccggtgaccgcccagctcccgcagaccaccgcctacggcgacgcctaccacggctactggcagcaggacatctactccctcaacgagaactacggcaccgccgacgacctcaaggccctctcctccgccctccacgagcgcggcatgtacctcatggtggacgtggtggccaaccacatgggctacgacggcgccggctcctccgtggactactccgtgttcaagccgttctcctcccaggactacttccacccgttctgcttcatccagaactacgaggaccagacccaggtggaggactgctggctcggcgacaacaccgtgtccctcccggacctcgacaccaccaaggacgtggtgaagaacgagtggtacgactgggtgggctccctcgtgtccaactactccatcgacggcctccgcatcgacaccgtgaagcacgtgcagaaggacttctggccgggctacaacaaggccgccggcgtgtactgcatcggcgaggtgctcgacgtggacccggcctacacctgcccgtaccagaacgtgatggacggcgtgctcaactacccgatctactacccgctcctcaacgccttcaagtccacctccggctcgatggacgacctctacaacatgatcaacaccgtgaagtccgactgcccggactccaccctcctcggcaccttcgtggagaaccacgacaacccgcgcttcgcctcctacaccaacgacatcgccctcgccaagaacgtggccgccttcatcatcctcaacgacggcatcccgatcatctacgccggccaggagcagcactacgccggcggcaacgacccggccaaccgcgaggccacctggctctccggctacccgaccgactccgagctgtacaagctcatcgcctccgccaacgccatccgcaactacgccatctccaaggacaccggcttcgtgacctacaagaactggccgatctacaaggacgacaccaccatcgccatgcgcaagggcaccgacggctcccagatcgtgaccatcctctccaacaagggcgcctccggcgactcctacaccctctccctctccggcgccggctacaccgccggccagcagctcaccgaggtgatcggctgcaccaccgtgaccgtgggctccgacggcaacgtgccggtgccgatggccggcggcctcccgcgcgtgctctacccgaccgagaagctcgccggctccaagatatgctcctcctccaagccggccaccctcgactcctggctctccaacgaggccaccgtggcccgcaccgccatcctcaacaacatcggcgccgacggcgcctgggtgtccggcgccgactccggcatcgtggtggcctccccgtccaccgacaacccggactacttctacacctggacccgcgactccggcatcgtgctcaagaccctcgtggacctcttccgcaacggcgacaccgacctcctctccaccatcgagcactacatctcctcccaggccatcatccagggcgtgtccaacccgtccggcgacctctcctccggcggcctcggcgagccgaagttcaacgtggacgagaccgcctacgccggctcctggggccgcccgcagcgcgacggcccggccctccgcgccaccgccatgatcggcttcggccagtggctcctcgacaacggctacacctccgccgccaccgagatcgtgtggccgctcgtgcgcaacgacctctcctacgtggcccagtactggaaccagaccggctacgacctctgggaggaggtgaacggctcctccttcttcaccatcgccgtgcagcaccgcgccctcgtggagggctccgccttcgccaccgccgtgggctcctcctgctcctggtgcgactcccaggccccgcagatcctctgctacctccagtccttctggaccggctcctacatcctcgccaacttcgactcctcccgctccggcaaggacaccaacaccctcctcggctccatccacaccttcgacccggaggccggctgcgacgactccaccttccagccgtgctccccgcgcgccctcgccaaccacaaggaggtggtggactccttccgctccatctacaccctcaacgacggcctctccgactccgaggccgtggccgtgggccgctacccggaggactcctactacaacggcaacccgtggttcctctgcaccctcgccgccgccgagcagctctacgacgccctctaccagtgggacaagcagggctccctggagatcaccgacgtgtccctcgacttcttcaaggccctctactccggcgccgccaccggcacctactcctcctcctcctccacctactcctccatcgtgtccgccgtgaagaccttcgccgacggcttcgtgtccatcgtggagacccacgccgcctccaacggctccctctccgagcagttcgacaagtccgacggcgacgagctgtccgcccgcgacctcacctggtcctacgccgccctcctcaccgccaacaaccgccgcaactccgtggtgccgccgtcctggggcgagacctccgcctcctccgtgccgggcacctgcgccgccacctccgcctccggcacctactcctccgtgaccgtgacctcctggccgtccatcgtggccaccggcggcaccaccaccaccgccaccaccaccggctccggcggcgtgacctccacctccaagaccaccaccaccgcctccaagacctccaccaccacctcctccacctcctgcaccaccccgaccgccgtggccgtgaccttcgacctcaccgccaccaccacctacggcgagaacatctacctcgtgggctccatctcccagctcggcgactgggagacctccgacggcatcgccctctccgccgacaagtacacctcctccaacccgccgtggtacgtgaccgtgaccctcccggccggcgagtccttcgagtacaagttcatccgcgtggagtccgacgactccgtggagtgggagtccgacccgaaccgcgagtacaccgtgccgcaggcctgcggcgagtccaccgccaccgtgaccgacacctggcgc

SEQ ID NO: 5 - DNA, 1320 bp, Artificial
  Synthetic
atggcgaagcacttggctgccatgtgctggtgcagcctcctagtgcttgtactgctctgcttgggctcccagctggcccaatcccaggtcctcttccaggggttcaactgggagtcgtggaagaagcaaggtgggtggtacaactacctcctggggcgggtggacgacatcgccgcgacgggggccacgcacgtctggctcccgcagccgtcgcactcggtggcgccgcaggggtacatgcccggccggctctacgacctggacgcgtccaagtacggcacccacgcggagctcaagtcgctcaccgcggcgttccacgccaagggcgtccagtgcgtcgccgacgtcgtgatcaaccaccgctgcgccgactacaaggacggccgcggcatctactgcgtcttcgagggcggcacgcccgacagccgcctcgactggggccccgacatgatctgcagcgacgacacgcagtactccaacgggcgcgggcaccgcgacacgggggccgacttcgccgccgcgcccgacatcgaccacctcaacccgcgcgtgcagcaggagctctcggactggctcaactggctcaagtccgacctcggcttcgacggctggcgcctcgacttcgccaagggctactccgccgccgtcgccaaggtgtacgtcgacagcaccgcccccaccttcgtcgtcgccgagatatggagctccctccactacgacggcaacggcgagccgtccagcaaccaggacgccgacaggcaggagctggtcaactgggcgcaggcggtgggcggccccgccgcggcgttcgacttcaccaccaagggcgtgctgcaggcggccgtccagggcgagctgtggcgcatgaaggacggcaacggcaaggcgcccgggatgatcggctggctgccggagaaggccgtcacgttcgtcgacaaccacgacaccggctccacgcagaactcgtggccattcccctccgacaaggtcatgcagggctacgcctatatcctcacgcacccaggaactccatgcatcttctacgaccacgttttcgactggaacctgaagcaggagatcagcgcgctgtctgcggtgaggtcaagaaacgggatccacccggggagcgagctgaacatcctcgccgccgacggggatctctacgtcgccaagattgacgacaaggtcatcgtgaagatcgggtcacggtacgacgtcgggaacctgatcccctcagacttccacgccgttgcccctggcaacaactactgcgtttgggagaagcacggtctgagagttccagcggggcggcaccactag